European Patent Application EP 4 725 964 A1, published April 15, 2026. Title: 结合Nectin-4的抗体及其用途. Applicant: 江苏迈威康新药研发有限公司. Application WO. The sequence listing filed with the application follows.

SEQUENCE LISTING (32 sequences)

SEQ ID NO: 1 - protein, 436 aa, synthetic construct
DVQLQESGPGLVKPSQSLSLTCSVTGYSITSNFYWNWIRQFPGNRLEWMGYISYDGSNNYNPSLKNRISISRDTSKNQFFLKLNSVTTEDTATYYCVRADYWGQGTLVTVSAAKTTPPSVYPLAPGSAAQTNSMVTLGCLVKGYFPEPVTVTWNSGSLSSGVHTFPAVLQSDLYTLSSSVTVPSSTWPSETVTCNVAHPASSTKVDKKIVPRDCGCKPCICTVPEVSSVFIFPPKPKDVLTITLTPKVTCVVVDISKDDPEVQFSWFVDDVEVHTAQTQPREEQFNSTFRSVSELPIMHQDWLNGKEFKCRVNSAAFPAPIEKTISKTKGRPKAPQVYTIPPPKEQMAKDKVSLTCMITDFFPEDITVEWQWNGQPAENYKNTQPIMDTDGSYFVYSKLNVQKSNWEAGNTFTCSVLHEGLHNHHTEKSLSHSPGK

SEQ ID NO: 2 - protein, 219 aa, synthetic construct
DTVMTQTPLSLPVSLGDQASISCRSSQSLESSDGHAYLNWYLQKPGQSPQLLIYRVSNRFSGVLHRFSGSGSGTDFTLKISRVEAEDLGVYFCLQFTHVPFTFGSGTKLEIKRADAAPTVSIFPPSSEQLTSGGASVVCFLNNFYPKDINVKWKIDGSERQNGVLNSWTDQDSKDSTYSMSSTLTLTKDEYERHNSYTCEATHKTSTSPIVKSFNRNEC

SEQ ID NO: 3 - protein, 112 aa, synthetic construct
DVQLQESGPGLVKPSQSLSLTCSVTGYSITSNFYWNWIRQFPGNRLEWMGYISYDGSNNYNPSLKNRISISRDTSKNQFFLKLNSVTTEDTATYYCVRADYWGQGTLVTVSA

SEQ ID NO: 4 - protein, 114 aa, synthetic construct
DTVMTQTPLSLPVSLGDQASISCRSSQSLESSDGHAYLNWYLQKPGQSPQLLIYRVSNRFSGVLHRFSGSGSGTDFTLKISRVEAEDLGVYFCLQFTHVPFTFGSGTKLEIKRA

SEQ ID NO: 5 - protein, 6 aa, synthetic construct
SNFYWN

SEQ ID NO: 6 - protein, 16 aa, synthetic construct
YISYDGSNNYNPSLKN

SEQ ID NO: 7 - skipped

SEQ ID NO: 8 - protein, 16 aa, synthetic construct
RSSQSLESSDGHAYLN

SEQ ID NO: 9 - protein, 7 aa, synthetic construct
RVSNRFS

SEQ ID NO: 10 - protein, 9 aa, synthetic construct
LQFTHVPFT

SEQ ID NO: 11 - protein, 443 aa, synthetic construct
SKSVEESGGRLVTPGTPLTLTCTVSGFSLSTYAMSWVRQAPGKGLEYIGIISGRGTTYYASWLKGRFTISKTSTTVDLKITSPTTEDTATYFCARDAGISDVYTGYFNLWGQGTLVTVSSGQPKAPSVFPLAPCCGDTPSSTVTLGCLVKGYLPEPVTVTWNSGTLTNGVRTFPSVRQSSGLYSLSSVVSVTSSSQPVTCNVAHPATNTKVDKTVAPSTCSKPTCPPPELLGGPSVFIFPPKPKDTLMISRTPEVTCVVVDVSQDDPEVQFTWYINNEQVRTARPPLREQQFNSTIRVVSTLPIAHQDWLRGKEFKCKVHNKALPAPIEKTISKARGQPLEPKVYTMGPPREELSSRSVSLTCMINGFYPSDISVEWEKNGKAEDNYKTTPAVLDSDGSYFLYSKLSVPTSEWQRGDVFTCSVMHEALHNHYTQKSISRSPGK

SEQ ID NO: 12 - protein, 217 aa, synthetic construct
QPVLAQLPSASAALGASAKLTCTLSSAHRTYTIAWYQQQQGEAPRYLMMLKSDGSYTKGTGVPDRFSGSSSGADRYLIISSVQAADEADYYCGADDSGGYVFGGGTQLTVTGQPAVTPSVILFPPSSEELKDNKATLVCLINDFYPGTVKVNWKADGTPVTQGVDTTQPSKQSNSKYAASSFLSLSANQWKSYQSVTCQVTHEGHTVEKSLAPAECS

SEQ ID NO: 13 - protein, 120 aa, synthetic construct
SKSVEESGGRLVTPGTPLTLTCTVSGFSLSTYAMSWVRQAPGKGLEYIGIISGRGTTYYASWLKGRFTISKTSTTVDLKITSPTTEDTATYFCARDAGISDVYTGYFNLWGQGTLVTVSS

SEQ ID NO: 14 - protein, 114 aa, synthetic construct
QPVLAQLPSASAALGASAKLTCTLSSAHRTYTIAWYQQQQGEAPRYLMMLKSDGSYTKGTGVPDRFSGSSSGADRYLIISSVQAADEADYYCGADDSGGYVFGGGTQLTVTGQP

SEQ ID NO: 15 - protein, 5 aa, synthetic construct
TYAMS

SEQ ID NO: 16 - protein, 16 aa, synthetic construct
IISGRGTTYYASWLKG

SEQ ID NO: 17 - protein, 14 aa, synthetic construct
DAGISDVYTGYFNL

SEQ ID NO: 18 - protein, 12 aa, synthetic construct
TLSSAHRTYTIA

SEQ ID NO: 19 - protein, 11 aa, synthetic construct
LKSDGSYTKGT

SEQ ID NO: 20 - protein, 9 aa, synthetic construct
GADDSGGYV

SEQ ID NO: 21 - protein, 448 aa, synthetic construct
SQSVEESGGRLVTPGTPLTLTCTVSGFSLSSYAMSWVRQAPGKGLEYIGIIGGRGTTYYAIWAKGRFTISKTSTTVDLKITSPTTEDTATYFCARDAGTTYVGTTYVATGYFNLWGQGTLVTVSSGQPKAPSVFPLAPCCGDTPSSTVTLGCLVKGYLPEPVTVTWNSGTLTNGVRTFPSVRQSSGLYSLSSVVSVTSSSQPVTCNVAHPATNTKVDKTVAPSTCSKPTCPPPELLGGPSVFIFPPKPKDTLMISRTPEVTCVVVDVSQDDPEVQFTWYINNEQVRTARPPLREQQFNSTIRVVSTLPIAHQDWLRGKEFKCKVHNKALPAPIEKTISKARGQPLEPKVYTMGPPREELSSRSVSLTCMINGFYPSDISVEWEKNGKAEDNYKTTPAVLDSDGSYFLYSKLSVPTSEWQRGDVFTCSVMHEALHNHYTQKSISRSPGK

SEQ ID NO: 22 - protein, 217 aa, synthetic construct
QPVLTQPPSASAALGASAKLTCTLSSAHKTYTIAWYQQQQGEAPRYLMILKSDGSYTRGTGVPDRFSGSSSGADRYLIISSVQADDEADYYCGADDSGGYVFGGGTQLTVTGQPAVTPSVILFPPSSEELKDNKATLVCLINDFYPGTVKVNWKADGTPVTQGVDTTQPSKQSNSKYAASSFLSLSANQWKSYQSVTCQVTHEGHTVEKSLAPAECS

SEQ ID NO: 23 - protein, 125 aa, synthetic construct
SQSVEESGGRLVTPGTPLTLTCTVSGFSLSSYAMSWVRQAPGKGLEYIGIIGGRGTTYYAIWAKGRFTISKTSTTVDLKITSPTTEDTATYFCARDAGTTYVGTTYVATGYFNLWGQGTLVTVSS

SEQ ID NO: 24 - protein, 114 aa, synthetic construct
QPVLTQPPSASAALGASAKLTCTLSSAHKTYTIAWYQQQQGEAPRYLMILKSDGSYTRGTGVPDRFSGSSSGADRYLIISSVQADDEADYYCGADDSGGYVFGGGTQLTVTGQP

SEQ ID NO: 25 - protein, 5 aa, synthetic construct
SYAMS

SEQ ID NO: 26 - protein, 16 aa, synthetic construct
IIGGRGTTYYAIWAKG

SEQ ID NO: 27 - protein, 19 aa, synthetic construct
DAGTTYVGTTYVATGYFNL

SEQ ID NO: 28 - protein, 12 aa, synthetic construct
TLSSAHKTYTIA

SEQ ID NO: 29 - protein, 11 aa, synthetic construct
LKSDGSYTRGT

SEQ ID NO: 30 - protein, 9 aa, synthetic construct
GADDSGGYV

SEQ ID NO: 31 - protein, 510 aa, synthetic construct
MPLSLGAEMWGPEAWLLLLLLLASFTGRCPAGELETSDVVTVVLGQDAKLPCFYRGDSGEQVGQVAWARVDAGEGAQELALLHSKYGLHVSPAYEGRVEQPPPPRNPLDGSVLLRNAVQADEGEYECRVSTFPAGSFQARLRLRVLVPPLPSLNPGPALEEGQGLTLAASCTAEGSPAPSVTWDTEVKGTTSSRSFKHSRSAAVTSEFHLVPSRSMNGQPLTCVVSHPGLLQDQRITHILHVSFLAEASVRGLEDQNLWHIGREGAMLKCLSEGQPPPSYNWTRLDGPLPSGVRVDGDTLGFPPLTTEHSGIYVCHVSNEFSSRDSQVTVDVLDPQEDSGKQVDLVSASVVVVGVIAALLFCLLVVVVVLMSRYHRRKAQQMTQKYEEELTLTRENSIRRLHSHHTDPRSQPEESVGLRAEGHPDSLKDNSSCSVMSEEPEGRSYSTLTTVREIETQTELLSPGSGRAEEEEDQDEGIKQAMNHFVQENGTLRAKPTGNGIYINGRGHLV

SEQ ID NO: 32 - protein, 318 aa, synthetic construct
GELETSDVVTVVLGQDAKLPCFYRGDSGEQVGQVAWARVDAGEGAQELALLHSKYGLHVSPAYEGRVEQPPPPRNPLDGSVLLRNAVQADEGEYECRVSTFPAGSFQARLRLRVLVPPLPSLNPGPALEEGQGLTLAASCTAEGSPAPSVTWDTEVKGTTSSRSFKHSRSAAVTSEFHLVPSRSMNGQPLTCVVSHPGLLQDQRITHILHVSFLAEASVRGLEDQNLWHIGREGAMLKCLSEGQPPPSYNWTRLDGPLPSGVRVDGDTLGFPPLTTEHSGIYVCHVSNEFSSRDSQVTVDVLDPQEDSGKQVDLVSAS